European Patent Application EP 4 700 120 A1, published February 25, 2026. Title: DON 분해 활성을 갖는 신규 폴리펩티드. Applicant: 씨제이제일제당 주식회사. The sequence listing filed with the application follows.

SEQUENCE LISTING (8 sequences)

SEQ ID NO: 1 - protein, 182 aa, Gossypium harknessii SPG
MGSLDSKESPANNPGLHSPPDEATKGYILQQTMFRIKDPKPALEFYSRVLGMSLLNKVDVPYMKMTLYMMGYEDVSSAPSDPVEKTIWTFGRPATMELTHFWGTENDPEFKGYHDGNSEPTGFGHIGITVDDMYKACERFESLGVEFVKKPGDGYAFIKDPDGYWIEIFDLNGIRAIVNNLA

SEQ ID NO: 2 - DNA, 546 bp, Gossypium harknessii SPG
  source 1..546: mol_type = genomic DNA
atggggtcccttgatagcaaagaatcgcccgctaataaccctggacttcatagtccccccgacgaggccacaaaaggctacatccttcaacaaactatgttccgcataaaagacccgaagccagcactggagttctattctagagtattggggatgtcattactgaacaaagtggatgtaccatacatgaaaatgaccctgtacatgatgggttacgaagatgtttcatctgccccaagcgatcccgtcgagaagactatttggacgttcggccgtcctgcaacgatggaactgacccatttttgggggaccgagaatgaccccgaatttaagggttaccatgacgggaactcagaacctaccggttttggccatattggtattactgtggatgatatgtataaagcgtgcgagcggtttgagagccttggtgttgaatttgttaaaaaaccaggagacggatatgcttttatcaaggacccggacggctactggattgagatttttgatttgaacggaatacgggctatcgtaaataacttagca

SEQ ID NO: 3 - protein, 182 aa, synthetic construct
MASSGPKESAANNPGLQTPPDEATKGYFMQQTMFRIKDPKVSLDFYSRVLGMSLLKRIDVPDMKFTLYFMGYEDVSSAPSDPIERTAWTFGRPATIELTHKWGTESDPEFKGYHNGNSEPRGFGHIGITVDDTYKACERFERLGVEFVKKPDDGYAFIKDPDGYWIEIFDLKNIRNVVNGVA

SEQ ID NO: 4 - DNA, 546 bp, synthetic construct
  source 1..546: mol_type = other DNA
atggcatcgtccgggccgaaagagtcggctgccaataatcctggcttgcaaactccacctgacgaggccactaagggttattttatgcaacagacaatgtttcgcattaaagaccctaaagtgtctttggacttctattcgcgcgtgcttggtatgagccttttgaaaagaattgacgtcccggatatgaagttcacgttatattttatgggatatgaagatgtaagtagtgcgccaagtgatccaatagagcggaccgcctggacatttggcagaccagcgacaatcgaattgacccataagtggggtaccgagagcgacccggagtttaaaggttaccataatggcaattctgaaccacggggtttcgggcacataggcatcacggtcgatgacacttacaaggcgtgtgagagattcgaacgtcttggggtagaatttgtgaaaaagccggatgacggctatgcgtttattaaagaccccgatggctactggatagagatatttgacttgaagaatatacgcaatgtggtaaatggagtcgct

SEQ ID NO: 5 - protein, 182 aa, synthetic construct
MASSGPKESAANNPGLQTPPDEATKGYFMQQTMFRIKDPKVSLDFYSRVLGMSLLKRIDVPDMKMTLYFMGYEDVSSAPSDPIERTAWTFGRPATIELTHKWGTESDPEFKGYHNGNSEPRGFGHIGITVDDTYKACERFERLGVEFVKKPDDGYAFIKDPDGYWIEIFDLKNIRNVVNGVA

SEQ ID NO: 6 - DNA, 546 bp, synthetic construct
  source 1..546: mol_type = other DNA
atggcatcgtccgggccgaaagagtcggctgccaataatcctggcttgcaaactccacctgacgaggccactaagggttattttatgcaacagacaatgtttcgcattaaagaccctaaagtgtctttggacttctattcgcgcgtgcttggtatgagccttttgaaaagaattgacgtcccggatatgaagatgacgttatattttatgggatatgaagatgtaagtagtgcgccaagtgatccaatagagcggaccgcctggacatttggcagaccagcgacaatcgaattgacccataagtggggtaccgagagcgacccggagtttaaaggttaccataatggcaattctgaaccacggggtttcgggcacataggcatcacggtcgatgacacttacaaggcgtgtgagagattcgaacgtcttggggtagaatttgtgaaaaagccggatgacggctatgcgtttattaaagaccccgatggctactggatagagatatttgacttgaagaatatacgcaatgtggtaaatggagtcgct

SEQ ID NO: 7 - DNA, 41 bp, synthetic construct
  source 1..41: mol_type = other DNA
cccggatatgaagatgacgttatattttatgggatatgaag

SEQ ID NO: 8 - DNA, 40 bp, synthetic construct
  source 1..40: mol_type = other DNA
acgtcatcttcatatccgggacgtcaattcttttcaaaag